European Patent Specification EP 3 535 394 B1, published April 12, 2023. Title: DNA plasmids for the Fast Generation of Homologous Recombination Vectors For Cell Line Development. Applicant: Temple University-Of The Commonwealth System of Higher Education Perez-Leal, Oscar. The sequence listing filed with the application follows.

SEQUENCE LISTING (2 sequences)

SEQ ID NO: 1 - DNA, 1802 bp, Artificial Sequence
  Fast-HDR donor plasmid backbone with linker peptide
  misc_feature (706)..(780): n is a, c, g, or t
  misc_feature (859)..(933): n is a, c, g, or t
ggtaccggcttactaaaagccagataacagtatgcgtatttgcgcgctgatttttgcggtataagaatatatactgatatgtatacccgaagtatgtcaaaaagaggtgtgctatgaagcagcgtattacagtgacagttgacagcgacagctatcagttgctcaaggcatatatgatgtcaatatctccggtctggtaagcacaaccatgcagaatgaagcccgtcgtctgcgtgccgaacgctggaaagcggaaaatcaggaagggatggctgaggtcgcccggtttattgaaatgaacggctcttttgctgacgagaacagggactggtgaaatgcagtttaaggtttacacctataaaagagagagccgttatcgtctgtttgtggatgtacagagtgatattattgacacgcccgggcgacggatggtgatccccctggccagtgcacgtctgctgtcagataaagtctcccgtgaactttacccggtggtgcatatcggggatgaaagctggcgcatgatgaccaccgatatggccagtgtgccggtctccgttatcggggaagaagtggctgatctcagccaccgcgaaaatgacatcaaaaacgccattaacctgatgttctggggaatataaatgtcaggctccgttatacacagccagtctgcaggtcgacggtacccaaggcggtggagaattcnnnnnnnnnnnnnnnnnnnnnnnnnnnnnnnnnnnnnnnnnnnnnnnnnnnnnnnnnnnnnnnnnnnnnnnnnnngaattcggatctggagcaacaaacttctcactactcaaacaagcaggtgacgtggaggagaatcccgggccttctagannnnnnnnnnnnnnnnnnnnnnnnnnnnnnnnnnnnnnnnnnnnnnnnnnnnnnnnnnnnnnnnnnnnnnnnnnntctagataaattcgtcagtagggttgtaaaggtttttcttttcctgagaaaacaaccttttgttttctcaggttttgctttttggcctttccctagcttttaaaaaaaaaaagcaaaagacgctggtggctggcactcctggtttccaggacggggttcaagtccctgcggtgtctttgcttggatccggcttactaaaagccagataacagtatgcgtatttgcgcgctgatttttgcggtataagaatatatactgatatgtatacccgaagtatgtcaaaaagaggtgtgctatgaagcagcgtattacagtgacagttgacagcgacagctatcagttgctcaaggcatatatgatgtcaatatctccggtctggtaagcacaaccatgcagaatgaagcccgtcgtctgcgtgccgaacgctggaaagcggaaaatcaggaagggatggctgaggtcgcccggtttattgaaatgaacggctcttttgctgacgagaacagggactggtgaaatgcagtttaaggtttacacctataaaagagagagccgttatcgtctgtttgtggatgtacagagtgatattattgacacgcccgggcgacggatggtgatccccctggccagtgcacgtctgctgtcagataaagtctcccgtgaactttacccggtggtgcatatcggggatgaaagctggcgcatgatgaccaccgatatggccagtgtgccggtctccgttatcggggaagaagtggctgatctcagccaccgcgaaaatgacatcaaaaacgccattaacctgatgttctggggaatataaatgtcaggctccgttatacacagccagtctgcaggtcgacggatcc

SEQ ID NO: 2 - DNA, 2227 bp, Artificial Sequence
  Fast-HDR donor plasmid backbone with internal promoter
  misc_feature (706)..(755): n is a, c, g, or t
  misc_feature (1309)..(1358): n is a, c, g, or t
ggtaccggcttactaaaagccagataacagtatgcgtatttgcgcgctgatttttgcggtataagaatatatactgatatgtatacccgaagtatgtcaaaaagaggtgtgctatgaagcagcgtattacagtgacagttgacagcgacagctatcagttgctcaaggcatatatgatgtcaatatctccggtctggtaagcacaaccatgcagaatgaagcccgtcgtctgcgtgccgaacgctggaaagcggaaaatcaggaagggatggctgaggtcgcccggtttattgaaatgaacggctcttttgctgacgagaacagggactggtgaaatgcagtttaaggtttacacctataaaagagagagccgttatcgtctgtttgtggatgtacagagtgatattattgacacgcccgggcgacggatggtgatccccctggccagtgcacgtctgctgtcagataaagtctcccgtgaactttacccggtggtgcatatcggggatgaaagctggcgcatgatgaccaccgatatggccagtgtgccggtctccgttatcggggaagaagtggctgatctcagccaccgcgaaaatgacatcaaaaacgccattaacctgatgttctggggaatataaatgtcaggctccgttatacacagccagtctgcaggtcgacggtacccaaggcggtggagaattcnnnnnnnnnnnnnnnnnnnnnnnnnnnnnnnnnnnnnnnnnnnnnnnnnngaattcaataaaagatctttattttcattagatctgtgtgttggttttttgtgtgtcgctacaatattttcctgaacggaagaataaataaaacttgtcctgtaaagaaaacccaggtaaaggaaagtggcagtccagactgcccggaagttcctggaggctaaggcctcacccccgtcgcttgataggacctgctgagccacatgactaaggcacgatcgcctccgcacgtgtaaaggtgctgggttccaagatggctgccccgccgcgaggcccgacttaagtatgtcacttccgcaccagcgagaaaggcggacccttcagccaatgaggccatagggcggggctaggccatgatgggctttcaaactacccaatagggcgtccgaactaaagcgcctacaaagtaacgtcacgtcgagttgcagagcgccggcaggcggggcagaggtggccaagccaatgcgatggctggggcggggtcggacgctctataagttgtcgataggcgggcactccgccctagattctaaggaccgccgccaccaccggtnnnnnnnnnnnnnnnnnnnnnnnnnnnnnnnnnnnnnnnnnnnnnnnnnntctagataaattcgtcagtagggttgtaaaggtttttcttttcctgagaaaacaaccttttgttttctcaggttttgctttttggcctttccctagcttttaaaaaaaaaaagcaaaagacgctggtggctggcactcctggtttccaggacggggttcaagtccctgcggtgtctttgcttggatccggcttactaaaagccagataacagtatgcgtatttgcgcgctgatttttgcggtataagaatatatactgatatgtatacccgaagtatgtcaaaaagaggtgtgctatgaagcagcgtattacagtgacagttgacagcgacagctatcagttgctcaaggcatatatgatgtcaatatctccggtctggtaagcacaaccatgcagaatgaagcccgtcgtctgcgtgccgaacgctggaaagcggaaaatcaggaagggatggctgaggtcgcccggtttattgaaatgaacggctcttttgctgacgagaacagggactggtgaaatgcagtttaaggtttacacctataaaagagagagccgttatcgtctgtttgtggatgtacagagtgatattattgacacgcccgggcgacggatggtgatccccctggccagtgcacgtctgctgtcagataaagtctcccgtgaactttacccggtggtgcatatcggggatgaaagctggcgcatgatgaccaccgatatggccagtgtgccggtctccgttatcggggaagaagtggctgatctcagccaccgcgaaaatgacatcaaaaacgccattaacctgatgttctggggaatataaatgtcaggctccgttatacacagccagtctgcaggtcgacggatcc